European Patent Application EP 4 793 271 A1, published August 19, 2026. Title: 神経保護剤. Applicant: 国立研究開発法人国立精神・神経医療研究センター. The sequence listing filed with the application follows.

SEQUENCE LISTING (2 sequences)

SEQ ID NO: 1 - DNA, 2097 bp, Homo sapiens
  source 1..2097: mol_type = other DNA
atgctggcggtgcctgggccagatgggggcggtggcacgggcccatggtgggctgcgggtggccgcgggccccgcgaagtgtcgccgggggcaggcaccgaggtgcaggacgccctggagcgcgcgctgccggagctgcagcaggccttgtccgcgctgaagcaggcgggcggcgcgcgggccgtgggcgccggcctggccgaggtcttccaactggtggaggaggcctggctgctgccggccgtgggccgcgaggtagcccagggtctgtgcgacgccatccgcctcgatggcggcctcgacctgctgttgcggctgctgcaggcgccggagttggagacgcgtgtgcaggccgcgcgcctgctggagcagatcctggtggctgagaaccgagaccgcgtggcgcgcattgggctgggcgtgatcctgaacctggcgaaggaacgcgaacccgtagagctggcgcggagcgtggcaggcatcttggagcacatgttcaagcattcggaggagacatgccagaggctggtggcggccggcggcctggacgcggtgctgtattggtgccgccgcacggaccccgcgctgctgcgccactgcgcgctggcgctgggcaactgcgcgctgcacgggggccaggcggtgcagcgacgcatggtagagaagcgcgcagccgagtggctcttcccgctcgccttctccaaggaggacgagctgcttcggctgcacgcctgcctcgcagtagcggtgttggcgactaacaaggaggtggagcgcgaggtggagcgctcgggcacgctggcgctcgtggagccgcttgtggcctcgctggaccctggccgcttcgcccgctgtctggtggacgccagcgacacaagccagggccgcgggcccgacgacctgcagcgcctcgtgccgttgctcgactctaaccgcttggaggcgcagtgcatcggggctttctacctctgcgccgaggctgccatcaagagcctgcaaggcaagaccaaggtgttcagcgacatcggcgccatccagagcctgaaacgcctggtttcctactctaccaatggcactaagtcggcgctggccaagcgcgcgctgcgcctgctgggcgaggaggtgccacggcccatcctgccctccgtgcccagctggaaggaggccgaggttcagacgtggctgcagcagatcggtttctccaagtactgcgagagcttccgggagcagcaggtggatggcgacctgcttctgcggctcacggaggaggaactccagaccgacctgggcatgaaatcgggcatcacccgcaagaggttctttagggagctcacggagctcaagaccttcgccaactattctacgtgcgaccgcagcaacctggcggactggctgggcagcctggacccgcgcttccgccagtacacctacggcctggtcagctgcggcctggaccgctccctgctgcaccgcgtgtctgagcagcagctgctggaagactgcggcatccacctgggcgtgcaccgcgcccgcatcctcacggcggccagagaaatgctacactccccgctgccctgtactggtggcaaacccagtggggacactccagatgtcttcatcagctaccgccggaactcaggttcccagctggccagtctcctgaaggtgcacctgcagctgcatggcttcagtgtcttcattgatgtggagaagctggaagcaggcaagttcgaggacaaactcatccagagtgtcatgggtgcccgcaactttgtgttggtgctatcacctggagcactggacaagtgcatgcaagaccatgactgcaaggattgggtgcataaggagattgtgactgctttaagctgcggcaagaacattgtgcccatcattgatggcttcgagtggcctgagccccaggtcctgcctgaggacatgcaggctgtgcttactttcaacggtatcaagtggtcccacgaataccaggaggccaccattgagaagatcatccgcttcctgcagggccgctcctcccgggactcatctgcaggctctgacaccagtttggagggtgctgcacccatgggtccaacctaa

SEQ ID NO: 2 - protein, 698 aa, Homo sapiens
MLAVPGPDGGGGTGPWWAAGGRGPREVSPGAGTEVQDALERALPELQQALSALKQAGGARAVGAGLAEVFQLVEEAWLLPAVGREVAQGLCDAIRLDGGLDLLLRLLQAPELETRVQAARLLEQILVAENRDRVARIGLGVILNLAKEREPVELARSVAGILEHMFKHSEETCQRLVAAGGLDAVLYWCRRTDPALLRHCALALGNCALHGGQAVQRRMVEKRAAEWLFPLAFSKEDELLRLHACLAVAVLATNKEVEREVERSGTLALVEPLVASLDPGRFARCLVDASDTSQGRGPDDLQRLVPLLDSNRLEAQCIGAFYLCAEAAIKSLQGKTKVFSDIGAIQSLKRLVSYSTNGTKSALAKRALRLLGEEVPRPILPSVPSWKEAEVQTWLQQIGFSKYCESFREQQVDGDLLLRLTEEELQTDLGMKSGITRKRFFRELTELKTFANYSTCDRSNLADWLGSLDPRFRQYTYGLVSCGLDRSLLHRVSEQQLLEDCGIHLGVHRARILTAAREMLHSPLPCTGGKPSGDTPDVFISYRRNSGSQLASLLKVHLQLHGFSVFIDVEKLEAGKFEDKLIQSVMGARNFVLVLSPGALDKCMQDHDCKDWVHKEIVTALSCGKNIVPIIDGFEWPEPQVLPEDMQAVLTFNGIKWSHEYQEATIEKIIRFLQGRSSRDSSAGSDTSLEGAAPMGPT